European Patent Application EP 4 317 422 A2, published February 7, 2024. Title: COMBINATORIAL CANCER IMMUNOTHERAPY. Applicant: Senti Biosciences, Inc. Application WO PCT/US2018/027492, filed April 13, 2018. The sequence listing filed with the application follows.

SEQUENCE LISTING (9 sequences)

SEQ ID NO: 1 - DNA, 588 bp, synthetic construct
  misc_feature 1..588: note = Synthetic polynucleotide
  source 1..588: mol_type = other DNA
gttgacattgattattgactagttattaatagtaatcaattacggggtcattagttcatagcccatatatggagttccgcgttacataacttacggtaaatggcccgcctggctgaccgcccaacgacccccgcccattgacgtcaataatgacgtatgttcccatagtaacgccaatagggactttccattgacgtcaatgggtggagtatttacggtaaactgcccacttggcagtacatcaagtgtatcatatgccaagtacgccccctattgacgtcaatgacggtaaatggcccgcctggcattatgcccagtacatgaccttatgggactttcctacttggcagtacatctacgtattagtcatcgctattaccatggtgatgcggttttggcagtacatcaatgggcgtggatagcggtttgactcacggggatttccaagtctccaccccattgacgtcaatgggagtttgttttggcaccaaaatcaacgggactttccaaaatgtcgtaacaactccgccccattgacgcaaatgggcggtaggcgtgtacggtgggaggtctatataagcagagctc

SEQ ID NO: 2 - DNA, 544 bp, synthetic construct
  misc_feature 1..544: note = Synthetic polynucleotide
  source 1..544: mol_type = other DNA
ggatctgcgatcgctccggtgcccgtcagtgggcagagcgcacatcgcccacagtccccgagaagttggggggaggggtcggcaattgaaccggtgcctagagaaggtggcgcggggtaaactgggaaagtgatgtcgtgtactggctccgcctttttcccgagggtgggggagaaccgtatataagtgcagtagtcgccgtgaacgttctttttcgcaacgggtttgccgccagaacacagctgaagcttcgaggggctcgcatctctccttcacgcgcccgccgccctacctgaggccgccatccacgccggttgagtcgcgttctgccgcctcccgcctgtggtgcctcctgaactgcgtccgccgtctaggtaagtttaaagctcaggtcgagaccgggcctttgtccggcgctcccttggagcctacctagactcagccggctctccacgctttgcctgaccctgcttgctcaactctacgtctttgtttcgttttctgttctgcgccgttacagatccaagctgtgaccggcgcctac

SEQ ID NO: 3 - DNA, 399 bp, synthetic construct
  misc_feature 1..399: note = Synthetic polynucleotide
  source 1..399: mol_type = other DNA
tttatttagtctccagaaaaaggggggaatgaaagaccccacctgtaggtttggcaagctaggatcaaggttaggaacagagagacagcagaatatgggccaaacaggatatctgtggtaagcagttcctgccccggctcagggccaagaacagttggaacagcagaatatgggccaaacaggatatctgtggtaagcagttcctgccccggctcagggccaagaacagatggtccccagatgcggtcccgccctcagcagtttctagagaaccatcagatgtttccagggtgccccaaggacctgaaatgaccctgtgccttatttgaactaaccaatcagttcgcttctcgcttctgttcgcgcgcttctgctccccgagctcaataaaagagccca

SEQ ID NO: 4 - DNA, 511 bp, synthetic construct
  misc_feature 1..511: note = Synthetic polynucleotide
  source 1..511: mol_type = other DNA
ggggttggggttgcgccttttccaaggcagccctgggtttgcgcagggacgcggctgctctgggcgtggttccgggaaacgcagcggcgccgaccctgggtctcgcacattcttcacgtccgttcgcagcgtcacccggatcttcgccgctacccttgtgggccccccggcgacgcttcctgctccgcccctaagtcgggaaggttccttgcggttcgcggcgtgccggacgtgacaaacggaagccgcacgtctcactagtaccctcgcagacggacagcgccagggagcaatggcagcgcgccgaccgcgatgggctgtggccaatagcggctgctcagcggggcgcgccgagagcagcggccgggaaggggcggtgcgggaggcggggtgtggggcggtagtgtgggccctgttcctgcccgcgcggtgttccgcattctgcaagcctccggagcgcacgtcggcagtcggctccctcgttgaccgaatcaccgacctctctccccag

SEQ ID NO: 5 - DNA, 408 bp, synthetic construct
  misc_feature 1..408: note = Synthetic polynucleotide
  source 1..408: mol_type = other DNA
gtaacgccattttgcaaggcatggaaaaataccaaaccaagaatagagaagttcagatcaagggcgggtacatgaaaatagctaacgttgggccaaacaggatatctgcggtgagcagtttcggccccggcccggggccaagaacagatggtcaccgcagtttcggccccggcccgaggccaagaacagatggtccccagatatggcccaaccctcagcagtttcttaagacccatcagatgtttccaggctcccccaaggacctgaaatgaccctgcgccttatttgaattaaccaatcagcctgcttctcgcttctgttcgcgcgcttctgcttcccgagctctataaaagagctcacaacccctcactcggcgcgccagtcctccgacagactgagtcgcccggg

SEQ ID NO: 6 - DNA, 344 bp, synthetic construct
  misc_feature 1..344: note = Synthetic polynucleotide
  source 1..344: mol_type = other DNA
ctgtggaatgtgtgtcagttagggtgtggaaagtccccaggctccccagcaggcagaagtatgcaaagcatgcatctcaattagtcagcaaccaggtgtggaaagtccccaggctccccagcaggcagaagtatgcaaagcatgcatctcaattagtcagcaaccatagtcccgcccctaactccgcccatcccgcccctaactccgcccagttccgcccattctccgccccatggctgactaattttttttatttatgcagaggccgaggccgcctctgcctctgagctattccagaagtagtgaggaggcttttttggaggcctaggcttttgcaaaaagct

SEQ ID NO: 7 - DNA, 1229 bp, synthetic construct
  misc_feature 1..1229: note = Synthetic polynucleotide
  source 1..1229: mol_type = other DNA
gcgccgggttttggcgcctcccgcgggcgcccccctcctcacggcgagcgctgccacgtcagacgaagggcgcaggagcgttcctgatccttccgcccggacgctcaggacagcggcccgctgctcataagactcggccttagaaccccagtatcagcagaaggacattttaggacgggacttgggtgactctagggcactggttttctttccagagagcggaacaggcgaggaaaagtagtcccttctcggcgattctgcggagggatctccgtggggcggtgaacgccgatgattatataaggacgcgccgggtgtggcacagctagttccgtcgcagccgggatttgggtcgcggttcttgtttgtggatcgctgtgatcgtcacttggtgagttgcgggctgctgggctggccggggctttcgtggccgccgggccgctcggtgggacggaagcgtgtggagagaccgccaagggctgtagtctgggtccgcgagcaaggttgccctgaactgggggttggggggagcgcacaaaatggcggctgttcccgagtcttgaatggaagacgcttgtaaggcgggctgtgaggtcgttgaaacaaggtggggggcatggtgggcggcaagaacccaaggtcttgaggccttcgctaatgcgggaaagctcttattcgggtgagatgggctggggcaccatctggggaccctgacgtgaagtttgtcactgactggagaactcgggtttgtcgtctggttgcgggggcggcagttatgcggtgccgttgggcagtgcacccgtacctttgggagcgcgcgcctcgtcgtgtcgtgacgtcacccgttctgttggcttataatgcagggtggggccacctgccggtaggtgtgcggtaggcttttctccgtcgcaggacgcagggttcgggcctagggtaggctctcctgaatcgacaggcgccggacctctggtgaggggagggataagtgaggcgtcagtttctttggtcggttttatgtacctatcttcttaagtagctgaagctccggttttgaactatgcgctcggggttggcgagtgtgttttgtgaagttttttaggcaccttttgaaatgtaatcatttgggtcaatatgtaattttcagtgttagactagtaaagcttctgcaggtcgactctagaaaattgtccgctaaattctggccgtttttggcttttttgttagac

SEQ ID NO: 8 - DNA, 6029 bp, synthetic construct
  misc_feature 1..6029: note = Synthetic polynucleotide
  source 1..6029: mol_type = other DNA
acgcgtgtagtcttatgcaatactcttgtagtcttgcaacatggtaacgatgagttagcaacatgccttacaaggagagaaaaagcaccgtgcatgccgattggtggaagtaaggtggtacgatcgtgccttattaggaaggcaacagacgggtctgacatggattggacgaaccactgaattgccgcattgcagagatattgtatttaagtgcctagctcgatacaataaacgggtctctctggttagaccagatctgagcctgggagctctctggctaactagggaacccactgcttaagcctcaataaagcttgccttgagtgcttcaagtagtgtgtgcccgtctgttgtgtgactctggtaactagagatccctcagacccttttagtcagtgtggaaaatctctagcagtggcgcccgaacagggacctgaaagcgaaagggaaaccagagctctctcgacgcaggactcggcttgctgaagcgcgcacggcaagaggcgaggggcggcgactggtgagtacgccaaaaattttgactagcggaggctagaaggagagagatgggtgcgagagcgtcagtattaagcgggggagaattagatcgcgatgggaaaaaattcggttaaggccagggggaaagaaaaaatataaattaaaacatatagtatgggcaagcagggagctagaacgattcgcagttaatcctggcctgttagaaacatcagaaggctgtagacaaatactgggacagctacaaccatcccttcagacaggatcagaagaacttagatcattatataatacagtagcaaccctctattgtgtgcatcaaaggatagagataaaagacaccaaggaagctttagacaagatagaggaagagcaaaacaaaagtaagaccaccgcacagcaagcggccactgatcttcagacctggaggaggagatatgagggacaattggagaagtgaattatataaatataaagtagtaaaaattgaaccattaggagtagcacccaccaaggcaaagagaagagtggtgcagagagaaaaaagagcagtgggaataggagctttgttccttgggttcttgggagcagcaggaagcactatgggcgcagcctcaatgacgctgacggtacaggccagacaattattgtctggtatagtgcagcagcagaacaatttgctgagggctattgaggcgcaacagcatctgttgcaactcacagtctggggcatcaagcagctccaggcaagaatcctggctgtggaaagatacctaaaggatcaacagctcctggggatttggggttgctctggaaaactcatttgcaccactgctgtgccttggaatgctagttggagtaataaatctctggaacagattggaatcacacgacctggatggagtgggacagagaaattaacaattacacaagcttaatacactccttaattgaagaatcgcaaaaccagcaagaaaagaatgaacaagaattattggaattagataaatgggcaagtttgtggaattggtttaacataacaaattggctgtggtatataaaattattcataatgatagtaggaggcttggtaggtttaagaatagtttttgctgtactttctatagtgaatagagttaggcagggatattcaccattatcgtttcagacccacctcccaaccccgaggggacccgacaggcccgaaggaatagaagaagaaggtggagagagagacagagacagatccattcgattagtgaacggatctcgacggtatcggttaacttttaaaagaaaaggggggattggggggtacagtgcaggggaaagaatagtagacataatagcaacagacatacaaactaaagaattacaaaaacaaattacaaaaatcaaaattttatctcgacatggtggcgaccggtagcgctagcggatcgataagcttgatatcgcctgcagccgaattccttgacttgggatccgcgtcaagtggagcaaggcaggtggacagtcctgcaggcatgcgtgactgactgaggccgcgactctagtttaaactgcgtgactgactctagaagatccggcagtgcggccgcgtcgacaatcaacctctggattacaaaatttgtgaaagattgactggtattcttaactatgttgctccttttacgctatgtggatacgctgctttaatgcctttgtatcatgctattgcttcccgtatggctttcattttctcctccttgtataaatcctggttgctgtctctttatgaggagttgtggcccgttgtcaggcaacgtggcgtggtgtgcactgtgtttgctgacgcaacccccactggttggggcattgccaccacctgtcagctcctttccgggactttcgctttccccctccctattgccacggcggaactcatcgccgcctgccttgcccgctgctggacaggggctcggctgttgggcactgacaattccgtggtgttgtcggggaaatcatcgtcctttccttggctgctcgcctgtgttgccacctggattctgcgcgggacgtccttctgctacgtcccttcggccctcaatccagcggaccttccttcccgcggcctgctgccggctctgcggcctcttccgcgtcttcgccttcgccctcagacgagtcggatctccctttgggccgcctccccgcctggtacctttaagaccaatgacttacaaggcagctgtagatcttagccactttttaaaagaaaaggggggactggaagggctaattcactcccaacgaaaataagatctgctttttgcttgtactgggtctctctggttagaccagatctgagcctgggagctctctggctaactagggaacccactgcttaagcctcaataaagcttgccttgagtgcttcaagtagtgtgtgcccgtctgttgtgtgactctggtaactagagatccctcagacccttttagtcagtgtggaaaatctctagcagtagtagttcatgtcatcttattattcagtatttataacttgcaaagaaatgaatatcagagagtgagaggaacttgtttattgcagcttataatggttacaaataaagcaatagcatcacaaatttcacaaataaagcatttttttcactgcattctagttgtggtttgtccaaactcatcaatgtatcttatcatgtctggctctagctatcccgcccctaactccgcccagttccgcccattctccgccccatggctgactaattttttttatttatgcagaggccgaggccgcctcggcctctgagctattccagaagtagtgaggaggcttttttggaggcctagacttttgcagagacggcccaaattcgtaatcatggtcatagctgtttcctgtgtgaaattgttatccgctcacaattccacacaacatacgagccggaagcataaagtgtaaagcctggggtgcctaatgagtgagctaactcacattaattgcgttgcgctcactgcccgctttccagtcgggaaacctgtcgtgccagctgcattaatgaatcggccaacgcgcggggagaggcggtttgcgtattgggcgctcttccgcttcctcgctcactgactcgctgcgctcggtcgttcggctgcggcgagcggtatcagctcactcaaaggcggtaatacggttatccacagaatcaggggataacgcaggaaagaacatgtgagcaaaaggccagcaaaaggccaggaaccgtaaaaaggccgcgttgctggcgtttttccataggctccgcccccctgacgagcatcacaaaaatcgacgctcaagtcagaggtggcgaaacccgacaggactataaagataccaggcgtttccccctggaagctccctcgtgcgctctcctgttccgaccctgccgcttaccggatacctgtccgcctttctcccttcgggaagcgtggcgctttctcatagctcacgctgtaggtatctcagttcggtgtaggtcgttcgctccaagctgggctgtgtgcacgaaccccccgttcagcccgaccgctgcgccttatccggtaactatcgtcttgagtccaacccggtaagacacgacttatcgccactggcagcagccactggtaacaggattagcagagcgaggtatgtaggcggtgctacagagttcttgaagtggtggcctaactacggctacactagaaggacagtatttggtatctgcgctctgctgaagccagttaccttcggaaaaagagttggtagctcttgatccggcaaacaaaccaccgctggtagcggtggtttttttgtttgcaagcagcagattacgcgcagaaaaaaaggatctcaagaagatcctttgatcttttctacggggtctgacgctcagtggaacgaaaactcacgttaagggattttggtcatgagattatcaaaaaggatcttcacctagatccttttaaattaaaaatgaagttttaaatcaatctaaagtatatatgagtaaacttggtctgacagttaccaatgcttaatcagtgaggcacctatctcagcgatctgtctatttcgttcatccatagttgcctgactccccgtcgtgtagataactacgatacgggagggcttaccatctggccccagtgctgcaatgataccgcgagacccacgctcaccggctccagatttatcagcaataaaccagccagccggaagggccgagcgcagaagtggtcctgcaactttatccgcctccatccagtctattaattgttgccgggaagctagagtaagtagttcgccagttaatagtttgcgcaacgttgttgccattgctacaggcatcgtggtgtcacgctcgtcgtttggtatggcttcattcagctccggttcccaacgatcaaggcgagttacatgatcccccatgttgtgcaaaaaagcggttagctccttcggtcctccgatcgttgtcagaagtaagttggccgcagtgttatcactcatggttatggcagcactgcataattctcttactgtcatgccatccgtaagatgcttttctgtgactggtgagtactcaaccaagtcattctgagaatagtgtatgcggcgaccgagttgctcttgcccggcgtcaatacgggataataccgcgccacatagcagaactttaaaagtgctcatcattggaaaacgttcttcggggcgaaaactctcaaggatcttaccgctgttgagatccagttcgatgtaacccactcgtgcacccaactgatcttcagcatcttttactttcaccagcgtttctgggtgagcaaaaacaggaaggcaaaatgccgcaaaaaagggaataagggcgacacggaaatgttgaatactcatactcttcctttttcaatattattgaagcatttatcagggttattgtctcatgagcggatacatatttgaatgtatttagaaaaataaacaaataggggttccgcgcacatttccccgaaaagtgccacctgacgtctaagaaaccattattatcatgacattaacctataaaaataggcgtatcacgaggccctttcgtctcgcgcgtttcggtgatgacggtgaaaacctctgacacatgcagctcccggagacggtcacagcttgtctgtaagcggatgccgggagcagacaagcccgtcagggcgcgtcagcgggtgttggcgggtgtcggggctggcttaactatgcggcatcagagcagattgtactgagagtgcaccatatgcggtgtgaaataccgcacagatgcgtaaggagaaaataccgcatcaggcgccattcgccattcaggctgcgcaactgttgggaagggcgatcggtgcgggcctcttcgctattacgccagctggcgaaagggggatgtgctgcaaggcgattaagttgggtaacgccagggttttcccagtcacgacgttgtaaaacgacggccagtgccaagctg

SEQ ID NO: 9 - DNA, 1179 bp, synthetic construct
  misc_feature 1..1179: note = Synthetic polynucleotide
  source 1..1179: mol_type = other DNA
ggctccggtgcccgtcagtgggcagagcgcacatcgcccacagtccccgagaagttggggggaggggtcggcaattgaaccggtgcctagagaaggtggcgcggggtaaactgggaaagtgatgccgtgtactggctccgcctttttcccgagggtgggggagaaccgtatataagtgcagtagtcgccgtgaacgttctttttcgcaacgggtttgccgccagaacacaggtaagtgccgtgtgtggttcccgcgggcctggcctctttacgggttatggcccttgcgtgccttgaattacttccacctggctgcagtacgtgattcttgatcccgagcttcgggttggaagtgggtgggagagttcgaggccttgcgcttaaggagccccttcgcctcgtgcttgagttgaggcctggcctgggcgctggggccgccgcgtgcgaatctggtggcaccttcgcgcctgtctcgctgctttcgataagtctctagccatttaaaatttttgatgacctgctgcgacgctttttttctggcaagatagtcttgtaaatgcgggccaagatctgcacactggtatttcggtttttggggccgcgggcggcgacggggcccgtgcgtcccagcgcacatgttcggcgaggcggggcctgcgagcgcgaccaccgagaatcggacgggggtagtctcaagctggccggcctgctctggtgcctgtcctcgcgccgccgtgtatcgccccgccccgggcggcaaggctggcccggtcggcaccagttgcgtgagcggaaagatggccgcttcccggtcctgctgcagggagctcaaaatggaggacgcggcgctcgggagagcgggcgggtgagtcacccacacaaaggaaaagggcctttccgtcctcagccgtcgcttcatgtgactccacggagtaccgggcgccgtccaggcacctcgattagttctcgagcttttggagtacgtcgtctttaggttggggggaggggttttatgcgatggagtttccccacactgagtgggtggagactgaagttaggccagcttggcacttgatgtaattctccttggaatttgccctttttgagtttggatcttggttcattctcaagcctcagacagtggttcaaagtttttttcttccatttcaggtgtcgtga